European Patent Application EP 4 413 992 A1, published August 14, 2024. Title: The Composition for Improving Activity of Natural Killer Cells. Applicant: KOREA RESEARCH INSTITUTE OF BIOSCIENCE AND BIOTECHNOLOGY. The sequence listing filed with the application follows.

SEQUENCE LISTING (2 sequences)

SEQ ID NO: 1 - protein, 13 aa, unidentified
GSKKVILDLPLVI

SEQ ID NO: 2 - DNA, 39 bp, unidentified
  source 1..39: mol_type = genomic DNA
agcagaacatccagcatggccagccgaaccagctctgag